European Patent Application EP 4 756 429 A2, published June 10, 2026. Title: Method and kit for the detection of Bovine Herpes Virus Type 1 (BoHV-1) antibodies. Applicant: IDEXX Laboratories, Inc. Application EP. The sequence listing filed with the application follows.

SEQUENCE LISTING (128 sequences)

SEQ ID NO: 1 - protein, 508 aa, Bovine Herpes Virus Type I
  REGION 1..508: note = full-length
MGPLGRAWLIAAIFAWALLSARRGLAEEAEASPSPPPSPSPTETESSAGTTGATPPTPNSPDATPEDSTPGATTPVGTPEPPSVSEHDPPVTNSTPPPAPPEDGRPGGAGNASRDGRPSGGGRPRPPRPSKAPPKERKWMLCEREAVAASYAEPLYVHCGVADNATGGARLELWFQRVGRFRSTRGDDEAVRNPFPRAPPVLLFVAQNGSIAYRSAELGDNYIFPSPADPRNLPLTVRSLTAATEGVYTWRRDMGTKSQRKVVTVTTHRAPAVSVEPQPALEGAGYAAVCRAAEYYPPRSTRLHWFRNGYPVEARHARDVFTVDDSGLFSRTSVLTLEDATPTAHPPNLRCDVSWFQSANMERRFYAAGTPAVYRPPELRVYFEGGEAVCEARCVPEGRVSLRWTVRDGIAPSRTEQTGVCAERPGLVNLRGVRLLSTTDGPVDYTCTATGYPAPLPEFSATATYDASPGLIGSPVLVSVVAVACGLGAVGLLLVAASCLRRKARARL

SEQ ID NO: 2 - protein, 508 aa, Bovine Herpes Virus Type I
  REGION 1..508: note = full-length with variants
  VARIANT 40: note = Xaa stands for Ser or Cys
  VARIANT 53: note = Xaa stands for Ala or Thr
  VARIANT 76: note = Xaa stands for Val or Gly
  VARIANT 128: note = Xaa stands for Arg or Gln
  VARIANT 136: note = Xaa stands for Glu or Gly
  VARIANT 138: note = Xaa stands for Lys or Glu
  VARIANT 143: note = Xaa stands for Glu or Lys
  VARIANT 168: note = Xaa stands for Gly or Asn
  VARIANT 205: note = Xaa stands for Val or Ala
  VARIANT 206: note = Xaa stands for Val or Ala
  VARIANT 220: note = Xaa stands for Asp or Gly
  VARIANT 238: note = Xaa stands for Arg or Cys
  VARIANT 256: note = Xaa stands for Thr or Ala
  VARIANT 278: note = Xaa stands for Gln or Arg
  VARIANT 282: note = Xaa stands for Glu or Gln
  VARIANT 294: note = Xaa stands for Glu or Lys
  VARIANT 304: note = Xaa stands for His or Arg
  VARIANT 356: note = Xaa stands for Phe or Tyr
  VARIANT 397: note = Xaa stands for Glu or Gly
  VARIANT 416: note = Xaa stands for Glu or Gly
  VARIANT 420: note = Xaa stands for Val or Ala
  VARIANT 472: note = Xaa stands for Ile or Val
MGPLGRAWLIAAIFAWALLSARRGLAEEAEASPSPPPSPXPTETESSAGTTGXTPPTPNSPDATPEDSTPGATTPXGTPEPPSVSEHDPPVTNSTPPPAPPEDGRPGGAGNASRDGRPSGGGRPRPPXPSKAPPKXRXWMLCXREAVAASYAEPLYVHCGVADNATGXARLELWFQRVGRFRSTRGDDEAVRNPFPRAPPVLLFXXQNGSIAYRSAELGXNYIFPSPADPRNLPLTVXSLTAATEGVYTWRRDMGXKSQRKVVTVTTHRAPAVSVEPXPALXGAGYAAVCRAAXYYPPRSTRLXWFRNGYPVEARHARDVFTVDDSGLFSRTSVLTLEDATPTAHPPNLRCDVSWXQSANMERRFYAAGTPAVYRPPELRVYFEGGEAVCEARCVPXGRVSLRWTVRDGIAPSRTXQTGXCAERPGLVNLRGVRLLSTTDGPVDYTCTATGYPAPLPEFSATATYDASPGLXGSPVLVSVVAVACGLGAVGLLLVAASCLRRKARARL

SEQ ID NO: 3 - protein, 449 aa, Bovine Herpes Virus Type I
  REGION 1..449: note = soluble domain
AEEAEASPSPPPSPSPTETESSAGTTGATPPTPNSPDATPEDSTPGATTPVGTPEPPSVSEHDPPVTNSTPPPAPPEDGRPGGAGNASRDGRPSGGGRPRPPRPSKAPPKERKWMLCEREAVAASYAEPLYVHCGVADNATGGARLELWFQRVGRFRSTRGDDEAVRNPFPRAPPVLLFVAQNGSIAYRSAELGDNYIFPSPADPRNLPLTVRSLTAATEGVYTWRRDMGTKSQRKVVTVTTHRAPAVSVEPQPALEGAGYAAVCRAAEYYPPRSTRLHWFRNGYPVEARHARDVFTVDDSGLFSRTSVLTLEDATPTAHPPNLRCDVSWFQSANMERRFYAAGTPAVYRPPELRVYFEGGEAVCEARCVPEGRVSLRWTVRDGIAPSRTEQTGVCAERPGLVNLRGVRLLSTTDGPVDYTCTATGYPAPLPEFSATATYDASPGLIGS

SEQ ID NO: 4 - protein, 449 aa, Bovine Herpes Virus Type I
  REGION 1..449: note = soluble domain with variants
  VARIANT 15: note = Xaa stands for Ser or Cys
  VARIANT 28: note = Xaa stands for Ala or Thr
  VARIANT 51: note = Xaa stands for Val or Gly
  VARIANT 103: note = Xaa stands for Arg or Gln
  VARIANT 111: note = Xaa stands for Glu or Gly
  VARIANT 113: note = Xaa stands for Lys or Glu
  VARIANT 118: note = Xaa stands for Glu or Lys
  VARIANT 143: note = Xaa stands for Gly or Asn
  VARIANT 180: note = Xaa stands for Val or Ala
  VARIANT 181: note = Xaa stands for Val or Ala
  VARIANT 195: note = Xaa stands for Asp or Gly
  VARIANT 213: note = Xaa stands for Arg or Cys
  VARIANT 231: note = Xaa stands for Thr or Ala
  VARIANT 253: note = Xaa stands for Gln or Arg
  VARIANT 257: note = Xaa stands for Glu or Gln
  VARIANT 269: note = Xaa stands for Glu or Lys
  VARIANT 279: note = Xaa stands for His or Arg
  VARIANT 331: note = Xaa stands for Phe or Tyr
  VARIANT 372: note = Xaa stands for Glu or Gly
  VARIANT 391: note = Xaa stands for Glu or Gly
  VARIANT 395: note = Xaa stands for Val or Ala
  VARIANT 447: note = Xaa stands for Ile or Val
AEEAEASPSPPPSPXPTETESSAGTTGXTPPTPNSPDATPEDSTPGATTPXGTPEPPSVSEHDPPVTNSTPPPAPPEDGRPGGAGNASRDGRPSGGGRPRPPXPSKAPPKXRXWMLCXREAVAASYAEPLYVHCGVADNATGXARLELWFQRVGRFRSTRGDDEAVRNPFPRAPPVLLFXXQNGSIAYRSAELGXNYIFPSPADPRNLPLTVXSLTAATEGVYTWRRDMGXKSQRKVVTVTTHRAPAVSVEPXPALXGAGYAAVCRAAXYYPPRSTRLXWFRNGYPVEARHARDVFTVDDSGLFSRTSVLTLEDATPTAHPPNLRCDVSWXQSANMERRFYAAGTPAVYRPPELRVYFEGGEAVCEARCVPXGRVSLRWTVRDGIAPSRTXQTGXCAERPGLVNLRGVRLLSTTDGPVDYTCTATGYPAPLPEFSATATYDASPGLXGS

SEQ ID NO: 5 - protein, 507 aa, Bovine Herpes Virus Type I
  REGION 1..507: note = soluble domain expression construct
METDTLLLWVLLLWVPGSTGDAAQPARRAEEAEASPSPPPSPSPTETESSAGTTGATPPTPNSPDATPEDSTPGATTPVGTPEPPSVSEHDPPVTNSTPPPAPPEDGRPGGAGNASRDGRPSGGGRPRPPRPSKAPPKERKWMLCEREAVAASYAEPLYVHCGVADNATGGARLELWFQRVGRFRSTRGDDEAVRNPFPRAPPVLLFVAQNGSIAYRSAELGDNYIFPSPADPRNLPLTVRSLTAATEGVYTWRRDMGTKSQRKVVTVTTHRAPAVSVEPQPALEGAGYAAVCRAAEYYPPRSTRLHWFRNGYPVEARHARDVFTVDDSGLFSRTSVLTLEDATPTAHPPNLRCDVSWFQSANMERRFYAAGTPAVYRPPELRVYFEGGEAVCEARCVPEGRVSLRWTVRDGIAPSRTEQTGVCAERPGLVNLRGVRLLSTTDGPVDYTCTATGYPAPLPEFSATATYDASPGLIGSGGSGGSSGLNDIFEAQKIEWHEGSHHHHHH

SEQ ID NO: 6 - protein, 15 aa, Bovine Herpes Virus Type I
AEEAEASPSPPPSPS

SEQ ID NO: 7 - protein, 15 aa, Bovine Herpes Virus Type I
EASPSPPPSPSPTET

SEQ ID NO: 8 - protein, 15 aa, Bovine Herpes Virus Type I
SPPPSPSPTETESSA

SEQ ID NO: 9 - protein, 15 aa, Bovine Herpes Virus Type I
SPSPTETESSAGTTG

SEQ ID NO: 10 - protein, 15 aa, Bovine Herpes Virus Type I
TETESSAGTTGATPP

SEQ ID NO: 11 - protein, 15 aa, Bovine Herpes Virus Type I
SSAGTTGATPPTPNS

SEQ ID NO: 12 - protein, 15 aa, Bovine Herpes Virus Type I
TTGATPPTPNSPDAT

SEQ ID NO: 13 - protein, 15 aa, Bovine Herpes Virus Type I
TPPTPNSPDATPEDS

SEQ ID NO: 14 - protein, 15 aa, Bovine Herpes Virus Type I
PNSPDATPEDSTPGA

SEQ ID NO: 15 - protein, 15 aa, Bovine Herpes Virus Type I
DATPEDSTPGATTPV

SEQ ID NO: 16 - protein, 15 aa, Bovine Herpes Virus Type I
EDSTPGATTPVGTPE

SEQ ID NO: 17 - protein, 15 aa, Bovine Herpes Virus Type I
PGATTPVGTPEPPSV

SEQ ID NO: 18 - protein, 15 aa, Bovine Herpes Virus Type I
TPVGTPEPPSVSEHD

SEQ ID NO: 19 - protein, 15 aa, Bovine Herpes Virus Type I
TPEPPSVSEHDPPVT

SEQ ID NO: 20 - protein, 15 aa, Bovine Herpes Virus Type I
PSVSEHDPPVTNSTP

SEQ ID NO: 21 - protein, 15 aa, Bovine Herpes Virus Type I
EHDPPVTNSTPPPAP

SEQ ID NO: 22 - protein, 15 aa, Bovine Herpes Virus Type I
PVTNSTPPPAPPEDG

SEQ ID NO: 23 - protein, 15 aa, Bovine Herpes Virus Type I
STPPPAPPEDGRPGG

SEQ ID NO: 24 - protein, 15 aa, Bovine Herpes Virus Type I
PAPPEDGRPGGAGNA

SEQ ID NO: 25 - protein, 15 aa, Bovine Herpes Virus Type I
EDGRPGGAGNASRDG

SEQ ID NO: 26 - protein, 15 aa, Bovine Herpes Virus Type I
PGGAGNASRDGRPSG

SEQ ID NO: 27 - protein, 15 aa, Bovine Herpes Virus Type I
GNASRDGRPSGGGRP

SEQ ID NO: 28 - protein, 15 aa, Bovine Herpes Virus Type I
RDGRPSGGGRPRPPR

SEQ ID NO: 29 - protein, 15 aa, Bovine Herpes Virus Type I
PSGGGRPRPPRPSKA

SEQ ID NO: 30 - protein, 15 aa, Bovine Herpes Virus Type I
GRPRPPRPSKAPPKE

SEQ ID NO: 31 - protein, 15 aa, Bovine Herpes Virus Type I
PPRPSKAPPKERKWM

SEQ ID NO: 32 - protein, 15 aa, Bovine Herpes Virus Type I
SKAPPKERKWMLCER

SEQ ID NO: 33 - protein, 15 aa, Bovine Herpes Virus Type I
PKERKWMLCEREAVA

SEQ ID NO: 34 - protein, 15 aa, Bovine Herpes Virus Type I
KWMLCEREAVAASYA

SEQ ID NO: 35 - protein, 15 aa, Bovine Herpes Virus Type I
CEREAVAASYAEPLY

SEQ ID NO: 36 - protein, 15 aa, Bovine Herpes Virus Type I
AVAASYAEPLYVHCG

SEQ ID NO: 37 - protein, 15 aa, Bovine Herpes Virus Type I
SYAEPLYVHCGVADN

SEQ ID NO: 38 - protein, 15 aa, Bovine Herpes Virus Type I
PLYVHCGVADNATGG

SEQ ID NO: 39 - protein, 15 aa, Bovine Herpes Virus Type I
HCGVADNATGGARLE

SEQ ID NO: 40 - protein, 15 aa, Bovine Herpes Virus Type I
ADNATGGARLELWFQ

SEQ ID NO: 41 - protein, 15 aa, Bovine Herpes Virus Type I
TGGARLELWFQRVGR

SEQ ID NO: 42 - protein, 15 aa, Bovine Herpes Virus Type I
RLELWFQRVGRFRST

SEQ ID NO: 43 - protein, 15 aa, Bovine Herpes Virus Type I
WFQRVGRFRSTRGDD

SEQ ID NO: 44 - protein, 15 aa, Bovine Herpes Virus Type I
VGRFRSTRGDDEAVR

SEQ ID NO: 45 - protein, 15 aa, Bovine Herpes Virus Type I
RSTRGDDEAVRNPFP

SEQ ID NO: 46 - protein, 15 aa, Bovine Herpes Virus Type I
GDDEAVRNPFPRAPP

SEQ ID NO: 47 - protein, 15 aa, Bovine Herpes Virus Type I
AVRNPFPRAPPVLLF

SEQ ID NO: 48 - protein, 15 aa, Bovine Herpes Virus Type I
PFPRAPPVLLFVAQN

SEQ ID NO: 49 - protein, 15 aa, Bovine Herpes Virus Type I
APPVLLFVAQNGSIA

SEQ ID NO: 50 - protein, 15 aa, Bovine Herpes Virus Type I
LLFVAQNGSIAYRSA

SEQ ID NO: 51 - protein, 15 aa, Bovine Herpes Virus Type I
AQNGSIAYRSAELGD

SEQ ID NO: 52 - protein, 15 aa, Bovine Herpes Virus Type I
SIAYRSAELGDNYIF

SEQ ID NO: 53 - protein, 15 aa, Bovine Herpes Virus Type I
RSAELGDNYIFPSPA

SEQ ID NO: 54 - protein, 15 aa, Bovine Herpes Virus Type I
LGDNYIFPSPADPRN

SEQ ID NO: 55 - protein, 15 aa, Bovine Herpes Virus Type I
YIFPSPADPRNLPLT

SEQ ID NO: 56 - protein, 15 aa, Bovine Herpes Virus Type I
SPADPRNLPLTVRSL

SEQ ID NO: 57 - protein, 15 aa, Bovine Herpes Virus Type I
PRNLPLTVRSLTAAT

SEQ ID NO: 58 - protein, 15 aa, Bovine Herpes Virus Type I
PLTVRSLTAATEGVY

SEQ ID NO: 59 - protein, 15 aa, Bovine Herpes Virus Type I
RSLTAATEGVYTWRR

SEQ ID NO: 60 - protein, 15 aa, Bovine Herpes Virus Type I
AATEGVYTWRRDMGT

SEQ ID NO: 61 - protein, 15 aa, Bovine Herpes Virus Type I
GVYTWRRDMGTKSQR

SEQ ID NO: 62 - protein, 15 aa, Bovine Herpes Virus Type I
WRRDMGTKSQRKVVT

SEQ ID NO: 63 - protein, 15 aa, Bovine Herpes Virus Type I
MGTKSQRKVVTVTTH

SEQ ID NO: 64 - protein, 15 aa, Bovine Herpes Virus Type I
SQRKVVTVTTHRAPA

SEQ ID NO: 65 - protein, 15 aa, Bovine Herpes Virus Type I
VVTVTTHRAPAVSVE

SEQ ID NO: 66 - protein, 15 aa, Bovine Herpes Virus Type I
TTHRAPAVSVEPQPA

SEQ ID NO: 67 - protein, 15 aa, Bovine Herpes Virus Type I
APAVSVEPQPALEGA

SEQ ID NO: 68 - protein, 15 aa, Bovine Herpes Virus Type I
SVEPQPALEGAGYAA

SEQ ID NO: 69 - protein, 15 aa, Bovine Herpes Virus Type I
QPALEGAGYAAVCRA

SEQ ID NO: 70 - protein, 15 aa, Bovine Herpes Virus Type I
EGAGYAAVCRAAEYY

SEQ ID NO: 71 - protein, 15 aa, Bovine Herpes Virus Type I
YAAVCRAAEYYPPRS

SEQ ID NO: 72 - protein, 15 aa, Bovine Herpes Virus Type I
CRAAEYYPPRSTRLH

SEQ ID NO: 73 - protein, 15 aa, Bovine Herpes Virus Type I
EYYPPRSTRLHWFRN

SEQ ID NO: 74 - protein, 15 aa, Bovine Herpes Virus Type I
PRSTRLHWFRNGYPV

SEQ ID NO: 75 - protein, 15 aa, Bovine Herpes Virus Type I
RLHWFRNGYPVEARH

SEQ ID NO: 76 - protein, 15 aa, Bovine Herpes Virus Type I
FRNGYPVEARHARDV

SEQ ID NO: 77 - protein, 15 aa, Bovine Herpes Virus Type I
YPVEARHARDVFTVD

SEQ ID NO: 78 - protein, 15 aa, Bovine Herpes Virus Type I
ARHARDVFTVDDSGL

SEQ ID NO: 79 - protein, 15 aa, Bovine Herpes Virus Type I
RDVFTVDDSGLFSRT

SEQ ID NO: 80 - protein, 15 aa, Bovine Herpes Virus Type I
TVDDSGLFSRTSVLT

SEQ ID NO: 81 - protein, 15 aa, Bovine Herpes Virus Type I
SGLFSRTSVLTLEDA

SEQ ID NO: 82 - protein, 15 aa, Bovine Herpes Virus Type I
SRTSVLTLEDATPTA

SEQ ID NO: 83 - protein, 15 aa, Bovine Herpes Virus Type I
VLTLEDATPTAHPPN

SEQ ID NO: 84 - protein, 15 aa, Bovine Herpes Virus Type I
EDATPTAHPPNLRCD

SEQ ID NO: 85 - protein, 15 aa, Bovine Herpes Virus Type I
PTAHPPNLRCDVSWF

SEQ ID NO: 86 - protein, 15 aa, Bovine Herpes Virus Type I
PPNLRCDVSWFQSAN

SEQ ID NO: 87 - protein, 15 aa, Bovine Herpes Virus Type I
RCDVSWFQSANMERR

SEQ ID NO: 88 - protein, 15 aa, Bovine Herpes Virus Type I
SWFQSANMERRFYAA

SEQ ID NO: 89 - protein, 15 aa, Bovine Herpes Virus Type I
SANMERRFYAAGTPA

SEQ ID NO: 90 - protein, 15 aa, Bovine Herpes Virus Type I
ERRFYAAGTPAVYRP

SEQ ID NO: 91 - protein, 15 aa, Bovine Herpes Virus Type I
YAAGTPAVYRPPELR

SEQ ID NO: 92 - protein, 15 aa, Bovine Herpes Virus Type I
TPAVYRPPELRVYFE

SEQ ID NO: 93 - protein, 15 aa, Bovine Herpes Virus Type I
YRPPELRVYFEGGEA

SEQ ID NO: 94 - protein, 15 aa, Bovine Herpes Virus Type I
ELRVYFEGGEAVCEA

SEQ ID NO: 95 - protein, 15 aa, Bovine Herpes Virus Type I
YFEGGEAVCEARCVP

SEQ ID NO: 96 - protein, 15 aa, Bovine Herpes Virus Type I
GEAVCEARCVPEGRV

SEQ ID NO: 97 - protein, 15 aa, Bovine Herpes Virus Type I
CEARCVPEGRVSLRW

SEQ ID NO: 98 - protein, 15 aa, Bovine Herpes Virus Type I
CVPEGRVSLRWTVRD

SEQ ID NO: 99 - protein, 15 aa, Bovine Herpes Virus Type I
GRVSLRWTVRDGIAP

SEQ ID NO: 100 - protein, 15 aa, Bovine Herpes Virus Type I
LRWTVRDGIAPSRTE

SEQ ID NO: 101 - protein, 15 aa, Bovine Herpes Virus Type I
VRDGIAPSRTEQTGV

SEQ ID NO: 102 - protein, 15 aa, Bovine Herpes Virus Type I
IAPSRTEQTGVCAER

SEQ ID NO: 103 - protein, 15 aa, Bovine Herpes Virus Type I
RTEQTGVCAERPGLV

SEQ ID NO: 104 - protein, 15 aa, Bovine Herpes Virus Type I
TGVCAERPGLVNLRG

SEQ ID NO: 105 - protein, 15 aa, Bovine Herpes Virus Type I
AERPGLVNLRGVRLL

SEQ ID NO: 106 - protein, 15 aa, Bovine Herpes Virus Type I
GLVNLRGVRLLSTTD

SEQ ID NO: 107 - protein, 15 aa, Bovine Herpes Virus Type I
LRGVRLLSTTDGPVD

SEQ ID NO: 108 - protein, 15 aa, Bovine Herpes Virus Type I
RLLSTTDGPVDYTCT

SEQ ID NO: 109 - protein, 15 aa, Bovine Herpes Virus Type I
TTDGPVDYTCTATGY

SEQ ID NO: 110 - protein, 15 aa, Bovine Herpes Virus Type I
PVDYTCTATGYPAPL

SEQ ID NO: 111 - protein, 15 aa, Bovine Herpes Virus Type I
TCTATGYPAPLPEFS

SEQ ID NO: 112 - protein, 15 aa, Bovine Herpes Virus Type I
TGYPAPLPEFSATAT

SEQ ID NO: 113 - protein, 15 aa, Bovine Herpes Virus Type I
APLPEFSATATYDAS

SEQ ID NO: 114 - protein, 15 aa, Bovine Herpes Virus Type I
EFSATATYDASPGLI

SEQ ID NO: 115 - protein, 13 aa, Bovine Herpes Virus Type I
TATYDASPGLIGS

SEQ ID NO: 116 - protein, 11 aa, Bovine Herpes Virus Type I
TPPTPNSPDAT

SEQ ID NO: 117 - protein, 7 aa, Bovine Herpes Virus Type I
PSVSEHD

SEQ ID NO: 118 - protein, 7 aa, Bovine Herpes Virus Type I
YAAVCRA

SEQ ID NO: 119 - protein, 11 aa, Bovine Herpes Virus Type I
TTDGPVDYTCT

SEQ ID NO: 120 - protein, 11 aa, Bovine Herpes Virus Type I
TATYDASPGLI

SEQ ID NO: 121 - protein, 15 aa, Bovine Herpes Virus Type I
  VARIANT 4: note = X stands for A or T
TTGXTPPTPNSPDAT

SEQ ID NO: 122 - protein, 15 aa, Bovine Herpes Virus Type I
  VARIANT 3: note = X stands for V or G
TPXGTPEPPSVSEHD

SEQ ID NO: 123 - protein, 15 aa, Bovine Herpes Virus Type I
  VARIANT 15: note = X stands for R or Q
RDGRPSGGGRPRPPX

SEQ ID NO: 124 - protein, 15 aa, Bovine Herpes Virus Type I
  VARIANT 1: note = X stands for Q or R
  VARIANT 5: note = X stands for E or Q
XPALXGAGYAAVCRA

SEQ ID NO: 125 - protein, 15 aa, Bovine Herpes Virus Type I
  VARIANT 9: note = X stands for E or K
YAAVCRAAXYYPPRS

SEQ ID NO: 126 - protein, 15 aa, Bovine Herpes Virus Type I
  VARIANT 15: note = X stands for I or V
EFSATATYDASPGLX

SEQ ID NO: 127 - protein, 13 aa, Bovine Herpes Virus Type I
  VARIANT 11: note = X stands for I or V
TATYDASPGLXGS

SEQ ID NO: 128 - protein, 11 aa, Bovine Herpes Virus Type I
  VARIANT 11: note = X stands for I or V
TATYDASPGLX